European Patent Specification EP 3 978 525 B1, published May 13, 2026. Title: MATERIALS AND METHODS FOR PERFORMING HISTOCHEMICAL ASSAYS FOR HUMAN PRO-EPIREGULIN AND AMPHIREGULIN. Applicant: Ventana Medical Systems, Inc. The sequence listing filed with the application follows.

SEQUENCE LISTING (52 sequences)

SEQ ID NO: 1 - protein, 169 aa, Homo sapiens
MTAGRRMEMLCAGRVPALLLCLGFHLLQAVLSTTVIPSCIPGESSDNCTALVQTEDNPRVAQVSITKCSSDMNGYCLHGQCIYLVDMSQNYCRCEVGYTGVRCEHFFLTVHQPLSKEYVALTVILIILFLITVVGSTYYFCRWYRNRKSKEPKKEYERVTSGDPELPQV

SEQ ID NO: 2 - protein, 5 aa, Oryctolagus cuniculus
RYGMS

SEQ ID NO: 3 - protein, 16 aa, Oryctolagus cuniculus
SINRTAYTYYATWAKG

SEQ ID NO: 4 - protein, 15 aa, Oryctolagus cuniculus
GLTYGGSDYDYDDAL

SEQ ID NO: 5 - protein, 29 aa, Oryctolagus cuniculus
QSVEESGGRLVTPGTPLTLTCTVSGFSLS

SEQ ID NO: 6 - protein, 14 aa, Oryctolagus cuniculus
WVRQAPGKGLEYIG

SEQ ID NO: 7 - protein, 30 aa, Oryctolagus cuniculus
RFTISRTSTTVDLRMTSLTTEDTATYFCAR

SEQ ID NO: 8 - protein, 11 aa, Oryctolagus cuniculus
WGPGTLVTVSS

SEQ ID NO: 9 - protein, 13 aa, Oryctolagus cuniculus
QASQSVYKNKNLA

SEQ ID NO: 10 - protein, 7 aa, Oryctolagus cuniculus
RASTLAS

SEQ ID NO: 11 - protein, 13 aa, Oryctolagus cuniculus
QGEFSCSTFDCIL

SEQ ID NO: 12 - protein, 22 aa, Oryctolagus cuniculus
QVLTQTPSSVSAAVGGTVTINC

SEQ ID NO: 13 - protein, 15 aa, Oryctolagus cuniculus
WYQQKPGQPPKLLIY

SEQ ID NO: 14 - protein, 32 aa, Oryctolagus cuniculus
GVSSRFKGSGSGTQFTLTISGVQCADAATYYC

SEQ ID NO: 15 - protein, 10 aa, Oryctolagus cuniculus
FGGGTEMVVK

SEQ ID NO: 16 - protein, 120 aa, Oryctolagus cuniculus
QSVEESGGRLVTPGTPLTLTCTVSGFSLSRYGMSWVRQAPGKGLEYIGSINRTAYTYYATWAKGRFTISRTSTTVDLRMTSLTTEDTATYFCARGLTYGGSDYDYDDALWGPGTLVTVSS

SEQ ID NO: 17 - protein, 112 aa, Oryctolagus cuniculus
QVLTQTPSSVSAAVGGTVTINCQASQSVYKNKNLAWYQQKPGQPPKLLIYRASTLASGVSSRFKGSGSGTQFTLTISGVQCADAATYYCQGEFSCSTFDCILFGGGTEMVVK

SEQ ID NO: 18 - protein, 5 aa, Oryctolagus cuniculus
TFAMA

SEQ ID NO: 19 - protein, 16 aa, Oryctolagus cuniculus
FISLSDATYYATWAKG

SEQ ID NO: 20 - protein, 14 aa, Oryctolagus cuniculus
VVGDSSGYPNTFHP

SEQ ID NO: 21 - protein, 29 aa, Oryctolagus cuniculus
KSVEESGGRLVTPGTPLTLTCTVSGIDLS

SEQ ID NO: 22 - protein, 14 aa, Oryctolagus cuniculus
WVRQAPGKGLEYIG

SEQ ID NO: 23 - protein, 31 aa, Oryctolagus cuniculus
RFTISKSSSTTVDLKIITPTAEDTATYFCAR

SEQ ID NO: 24 - protein, 11 aa, Oryctolagus cuniculus
WGPGTLVTVSS

SEQ ID NO: 25 - protein, 13 aa, Oryctolagus cuniculus
QASQSIHNSDFLA

SEQ ID NO: 26 - protein, 13 aa, Oryctolagus cuniculus
QASQNIHNSDFLA

SEQ ID NO: 27 - protein, 7 aa, Oryctolagus cuniculus
RASKLPS

SEQ ID NO: 28 - protein, 12 aa, Oryctolagus cuniculus
QGTYYSGGWYFT

SEQ ID NO: 29 - protein, 22 aa, Oryctolagus cuniculus
QVLTQTPSPVSAAVGGTVTINC

SEQ ID NO: 30 - protein, 15 aa, Oryctolagus cuniculus
WYQQKPGQPPKLLIY

SEQ ID NO: 31 - protein, 32 aa, Oryctolagus cuniculus
GVPSRFKGSGSGTQFTLTISDLECDDAATYYC

SEQ ID NO: 32 - protein, 10 aa, Oryctolagus cuniculus
FGGGTEVVVK

SEQ ID NO: 33 - protein, 120 aa, Oryctolagus cuniculus
KSVEESGGRLVTPGTPLTLTCTVSGIDLSTFAMAWVRQAPGKGLEYIGFISLSDATYYATWAKGRFTISKSSSTTVDLKIITPTAEDTATYFCARVVGDSSGYPNTFHPWGPGTLVTVSS

SEQ ID NO: 34 - protein, 111 aa, Oryctolagus cuniculus
QVLTQTPSPVSAAVGGTVTINCQASQSIHNSDFLAWYQQKPGQPPKLLIYRASKLPSGVPSRFKGSGSGTQFTLTISDLECDDAATYYCQGTYYSGGWYFTFGGGTEVVVK

SEQ ID NO: 35 - protein, 111 aa, Oryctolagus cuniculus
QVLTQTPSPVSAAVGGTVTINCQASQNIHNSDFLAWYQQKPGQPPKLLIYRASKLPSGVPSRFKGSGSGTQFTLTISDLECDDAATYYCQGTYYSGGWYFTFGGGTEVVVK

SEQ ID NO: 36 - protein, 252 aa, Homo sapiens
MRAPLLPPAPVVLSLLILGSGHYAAGLDLNDTYSGKREPFSGDHSADGFEVTSRSEMSSGSEISPVSEMPSSSEPSSGADYDYSEEYDNEPQIPGYIVDDSVRVEQVVKPPQNKTESENTSDKPKRKKKGGKNGKNRRNRKKKNPCNAEFQNFCIHGECKYIEHLEAVTCKCQQEYFGERCGEKSMKTHSMIDSSLSKIALAAIAAFMSAVILTAVAVITVQLRRQYVRKYEGEAEERKKLRQENGNVHAIA

SEQ ID NO: 37 - protein, 5 aa, Oryctolagus cuniculus
SYAIS

SEQ ID NO: 38 - protein, 17 aa, Oryctolagus cuniculus
FIVGSSGSAYYASWAKS

SEQ ID NO: 39 - protein, 8 aa, Oryctolagus cuniculus
GLYSGGNY

SEQ ID NO: 40 - protein, 29 aa, Oryctolagus cuniculus
QSLEESRGGLIKPGGTLTLTCTVSGFSLS

SEQ ID NO: 41 - protein, 14 aa, Oryctolagus cuniculus
WVRQAPGNGLEWIG

SEQ ID NO: 42 - protein, 32 aa, Oryctolagus cuniculus
RSTITRDTNLNTVTLKMTSLTAADTATYFCAK

SEQ ID NO: 43 - protein, 11 aa, Oryctolagus cuniculus
WGPGTLVTVSS

SEQ ID NO: 44 - protein, 13 aa, Oryctolagus cuniculus
QSSQSVDENNYLS

SEQ ID NO: 45 - protein, 7 aa, Oryctolagus cuniculus
RASTLES

SEQ ID NO: 46 - protein, 11 aa, Oryctolagus cuniculus
LGGYSGYSDDG

SEQ ID NO: 47 - protein, 22 aa, Oryctolagus cuniculus
AVLTQTPSPVSAAVGGTVSISC

SEQ ID NO: 48 - protein, 15 aa, Oryctolagus cuniculus
WFQQKPGQPPKLLIY

SEQ ID NO: 49 - protein, 32 aa, Oryctolagus cuniculus
GVPSRFSGSGSGTQFTLTVSGVQCDDAATYYC

SEQ ID NO: 50 - protein, 10 aa, Oryctolagus cuniculus
FGGGTEVVVK

SEQ ID NO: 51 - protein, 116 aa, Oryctolagus cuniculus
QSLEESRGGLIKPGGTLTLTCTVSGFSLSSYAISWVRQAPGNGLEWIGFIVGSSGSAYYASWAKSRSTITRDTNLNTVTLKMTSLTAADTATYFCAKGLYSGGNYWGPGTLVTVSS

SEQ ID NO: 52 - protein, 110 aa, Oryctolagus cuniculus
AVLTQTPSPVSAAVGGTVSISCQSSQSVDENNYLSWFQQKPGQPPKLLIYRASTLESGVPSRFSGSGSGTQFTLTVSGVQCDDAATYYCLGGYSGYSDDGFGGGTEVVVK